European Patent Application EP 4 477 738 A1, published December 18, 2024. Title: Engineered yeast strain with mitochondrial -targeted reductive tca pathway for high succinic acid production, construction method therefor and use thereof. Applicant: Shenghong Holding Group Co.Ltd. Application CN 2022/143484, filed December 29, 2022. The sequence listing filed with the application follows.

SEQUENCE LISTING (48 sequences)

SEQ ID NO: 1 - DNA, 3420 bp, synthetic construct
  source 1..3420: mol_type = other DNA
atggtggacggtcgatcttccgcctccatcgtcgccgtcgaccccgagcgagccgctcgagagcgagacgctgccgctcgagccctgctgcaggactcccctctgcacaccaccatgcagtacgccacctccggcctggagctgaccgtcccttacgccctgaaggtcgtcgcctccgccgacaccttcgaccgagccaaggaggtcgccgacgaggtgctgcgatgcgcctggcagctggccgacaccgtgctgaactctttcaaccccaactctgaggtctctctggtcggtcgactgcccgtcggccagaagcaccagatgtccgcccccctgaagcgagtcatggcctgttgccagcgagtctacaactcctccgccggttgtttcgacccctctaccgcccccgtggccaaggctctgcgagagattgccctgggtaaagagcgaaacaacgcctgcctggaggccctgacccaggcctgtaccctgcccaactccttcgtgattgacttcgaggccggcaccatctctcgaaagcacgagcacgcctctctggacctgggcggtgtctccaagggttacattgtggactacgtgatcgacaacatcaacgccgccggcttccagaacgtcttcttcgactggggcggcgactgccgagcctctggtatgaacgcccgaaacaccccctgggtcgtgggcattacccgacccccctccctggacatgctgcccaacccccccaaggaggcctcctacatctccgtgatctccctggacaacgaggccctggccacctctggtgactacgagaacctgatctacaccgccgacgacaagcccctgacctgtacctacgactggaagggcaaggagctgatgaagccctctcagtctaacatcgcccaggtctctgtcaagtgttactccgccatgtacgccgacgccctggccactgcctgtttcattaagcgagaccccgccaaggtccgacagctgctggacggttggcgatacgtccgagacaccgtccgagactaccgagtctacgtccgagagaacgagcgagtcgccaagatgttcgagattgccaccgaggacgccgagatgcgaaagcgacgaatctctaacaccctgcccgcccgagtcatcgtggtcggtggtggcctggccggtctgtccgctgctattgaggccgccggttgtggcgcccaggtggttctgatggagaaggaggccaagctgggtggtaactctgccaaggccacctccggaattaacggttggggcacccgagcccaggccaaggcttccattgtggacggtggcaagtacttcgagcgagacacctacaagtccggtatcggtggtaacaccgaccccgccctggtcaagaccctgtccatgaagtctgccgacgccattggctggctgacctccctgggtgtccccctgaccgtgctgtcccagctgggcggacactcccgaaagcgaacccaccgagcccccgacaagaaggacggcacccccctgcccattggcttcaccattatgaagaccctggaggaccacgtccgaggcaacctgtctggccgaatcaccatcatggagaactgctccgtcacctccctgctgtccgagaccaaggagcgacccgacggcaccaagcagatccgagtcaccggtgtggagttcacccaggccggctccggtaaaaccaccatcctggccgacgccgtgatcctggccaccggaggtttctccaacgacaagaccgccgactccctgctgcgagagcacgcccctcacctggtcaacttccccaccaccaacggtccctgggccaccggagacggtgtcaagctggcccagcgactgggtgcccagctggtcgacatggacaaggtccagctgcaccccaccggtctgattaaccccaaggaccccgccaaccccaccaagttcctgggccccgaggccctgcgaggctctggtggtgtgctgctgaacaagcagggcaagcgattcgtgaacgagctggacctgcgatctgtcgtctccaaggccatcatggagcagggtgccgagtaccccggttccggtggttccatgttcgcctactgtgtcctgaacgccgccgcccagaagctgttcggcgtctcttcccacgagttctactggaagaagatgggcctgttcgtcaaggccgacaccatgcgagacctggccgccctgattggttgccccgtggagtccgtgcagcagaccctggaggagtacgagcgactgtccatttcccagcgatcttgccccattacccgaaagtccgtgtacccctgcgtcctgggcaccaagggcccctactacgtcgccttcgtcaccccctccattcactacaccatgggtggttgcctgatttccccctccgccgagatccagatgaagaacacctcctctcgagcccccctgtcccactccaaccccatcctgggtctgttcggtgccggcgaggtgaccggcggtgtccatggtggcaaccgactgggcggcaactccctgctggagtgtgtcgtcttcggccgaatcgccggcgaccgagcctctaccatcctgcagcgaaagtcctccgccctgtctttcaaggtgtggaccaccgtggtcctgcgagaggtccgagagggcggtgtgtacggcgccggttcccgagtgctgcgattcaacctgcccggcgccctgcagcgatctggcctttctctgggccagttcattgccatccgaggcgactgggacggtcagcagctgatcggttactactctcccatcaccctgcccgacgacctgggtatgatcgacattctggcccgatctgacaagggcaccctgcgagagtggatttctgccctggagcccggcgacgccgtcgagatgaaggcctgtggcggtctggtcatcgagcgacgactgtctgacaagcacttcgtgttcatgggccacatcatcaacaagctgtgtctgatcgccggcggtaccggcgtcgcccctatgcttcagatcattaaggccgccttcatgaagcccttcattgacaccctggagtctgtgcacctgatctacgccgccgaggacgtcaccgagctgacctaccgagaggtgctggaggagcgacgacgagagtcccgaggcaagttcaagaagaccttcgtgctgaaccgacccccccccctgtggaccgacggagttggattcattgaccgaggtattctgaccaaccacgtccagcccccctctgacaacctgctggtggccatttgcggcccccccgtcatgcagcgaatcgtgaaggccaccctgaagaccctgggctacaacatgaacctggtgcgaaccgtggacgagaccgagccctctggctcctaa

SEQ ID NO: 2 - DNA, 1506 bp, synthetic construct
  source 1..1506: mol_type = other DNA
atgatccgatccgtgcgacgagtgttcatctacgtgtctatcttcgtgctgatcattgtgctgaagcgaaccctgtctggcaccgaccagacctctatgaagcagcccgtggtggtgatcggctctggcctggccggcctgaccacctctaaccgactgatctctaagtacagaatccccgtggtgctgctggacaaggctgcctctatcggcggcaactctatcaaggcctcttctggcatcaacggcgcccacaccgacactcagcagaacctgaaggtgatggatacccctgagctgttcctgaaggacaccctgcactctgccaagggccgaggcgtgccctctctgatggacaagctgaccaaggaatctaagtctgccatccgatggctgcagaccgagttcgacctgaagctggacctgctcgcccagctcggcggacactctgtgccccgaactcaccgatcttccggcaagctgcctcctggcttcgagattgtgcaggccctgtctaagaagctcaaggacatctcttccaaggactctaacctggtgcagatcatgctgaactctgaggtggtggacatcgagctggacaaccagggccacgtgaccggcgtggtgtacatggacgagaacggcaaccgaaagatcatgaagtctcaccacgtcgtgttctgctctggcggcttcggatactctaaggaaatgctgaaggaatactctcccaacctgattcatctgcccaccaccaacggcaagcagaccaccggcgacggccagaagatcctgtccaagctgggagccgagctgatcgacatggaccaggtccaggtgcaccccaccggcttcatcgaccccaacgaccgagagaacaactggaagttcctggccgctgaggccctgcgaggactcggcggaatcctgctgcaccctaccactggccgacgattcaccaacgagctgtctacccgagacaccgtgaccatggaaatccagtctaagtgccccaagaacgacaacagagccctgctggtgatgtctgacaaggtgtacgagaactacaccaacaacatcaacttctacatgtccaagaacctgatcaagaaggtgtctatcaacgacctgatccgacagtacgacctgcagaccactgcctccgagctggtcaccgagctgaagtcttactctgacgtgaacaccaaggacaccttcgaccgacctctgatcatcaacgccttcgacaaggacatttctaccgagtctaccgtgtacgtcggcgaggtgacccctgtggtgcacttcaccatgggcggagtgaagatcaacgagaagtctcaggtgattaagaagaactccgagtctgtcctgtctaacggcatcttcgctgctggcgaggtgtctggcggagtgcacggcgccaaccgactcggaggatcttccctgcttgagtgcgtggtgttcggcaagaccgccgctgacaacattgccaagctgtactaa

SEQ ID NO: 3 - DNA, 1791 bp, synthetic construct
  source 1..1791: mol_type = other DNA
atgaagaagatgaacctggccgtctgtatcgctaccctgatgggcaccgccggactcatgggaaccgccgtggccgccgacaacctggctgagttccacgtgcagaaccaggaatgcgactcttgtcacacccctgacggcgagctgtctaacgactctctgacctacgagaacacccagtgcgtgtcttgccacggcaccctggccgaggtggccgagactaccaagcacgagcactacaacgcccacgcctctcacttccccggcgaggtcgcctgcacctcttgccactctgcccacgagaagtctatggtgtactgcgactcctgccactctttcgacttcaacatgccctacgccaagaagtggctgcgggacgagcccaccattgccgagctggccaaggacaagtctgagcgacaggccgctctggcctctgctccccacgacaccgtggacgtggtggtggtcggctctggcggagccggcttctctgccgccatctctgccaccgactctggcgccaaggtgatcctgatcgagaaggaacccgtgatcggcggcaacgccaagctggccgctggcggcatgaacgccgcctggaccgaccagcagaaggccaagaagattaccgactctcccgagctgatgttcgaggacaccatgaagggcggccagaacatcaacgaccccgctctggtgaaggtgctgtcctctcactctaaggactctgtggactggatgaccgccatgggagccgacctgaccgacgtgggcatgatgggcggagcctctgtgaacagagcccaccgacctaccggcggagctggcgtgggagcccatgtggtgcaggtcctgtacgacaacgccgtgaagcgaaacatcgacctgcgaatgaacacccgaggcatcgaggtgctgaaggacgacaagggcaccgtgaagggcatcctggtcaagggcatgtacaagggctactactgggtgaaggccgacgccgtgatcctggccaccggcggcttcgccaagaacaacgagcgagtggctaagctggacccctcgctgaagggcttcatctctaccaaccagcctggcgccgtcggcgacggactggacgtcgccgagaacgctggtggcgccctgaaggacatgcagtacatccaggctcaccccactctgtctgtcaagggcggcgtgatggtgaccgaggccgtgcgaggcaacggcgccatcctggtgaaccgagagggcaagcgattcgtgaacgagatcactacccgagacaaggcctccgccgccattctggcccagaccggcaagtctgcctacctgatcttcgacgactctgtgcgaaagtctctgtctaagatcgacaagtacatcggcctgggcgtcgcccctaccgctgactccctggtgaagctgggcaagatggaaggcatcgacggcaaggccctgaccgagactgtggcccgatacaactctctggtgtcgtctggcaaggacaccgacttcgagcgacccaacctgcctcgggctctgaacgagggcaactactacgccattgaggtgacccctggcgtgcaccacaccatgggaggcgtgatgatcgacaccaaggccgaggtcatgaacgctaagaagcaggtcatccccggcctgtacggcgctggcgaggtgaccggcggtgtgcacggcgccaaccgactcggaggaaacgccatctccgacatcatcaccttcggccgactggccggcgaggaagccgccaagtactctaagaagaactaa

SEQ ID NO: 4 - DNA, 987 bp, synthetic construct
  source 1..987: mol_type = other DNA
atgaactctccccagaacgtgtctaccaagaaggtgaccgtcaccggcgctgccggccagatctcttactctctgctgtggcgaatcgccaacggcgaggtgttcggcaccgacactcccgtcgagctgaagctgctcgagattccccaggctctcggcggagccgagggcgtcgccatggaactgctggactctgctttccctctgctgcgaaacatcaccatcaccgccgacgccaacgaggccttcgacggcgccaacgccgccttcctggtgggcgctaagccccgaggcaagggcgaagaacgagccgacctgctggccaacaacggcaagatcttcggaccccaaggcaaggccatcaacgacaacgccgctgacgacatccgagtgctggtggtgggcaaccccgccaacaccaacgctctgatcgcctctgccgctgctcccgacgtgcccgcctctcgattcaacgccatgatgcgactggaccacaaccgagccatctctcagctggccaccaagctcggacgaggctctgccgagttcaacaacatcgtggtgtggggcaaccactctgccactcagttccccgacatcacctacgccaccgtcggcggcgagaaggtcaccgacctggtggaccacgactggtacgtggaagagttcattccccgagtggccaaccgaggcgccgagatcatcgaggtgcgaggcaagtcctccgccgcttctgccgcctcttccgccatcgaccacatgcgagactgggtgcagggaaccgaggcctggtcctccgctgctatcccctctaccggcgcctacggcatccccgagggcatcttcgtgggactgcccaccgtgtctcgaaacggcgagtgggagatcgtcgagggactcgagatctctgacttccagcgagcccgaatcgacgctaacgcccaagagctgcaggccgagcgagaggccgtgcgagatctgctgtaa

SEQ ID NO: 5 - DNA, 1404 bp, synthetic construct
  source 1..1404: mol_type = other DNA
atgaacaccgtgcgatctgagaaggactctatgggcgccatcgacgtgcccgccgacaagctgtggggcgctcagacccagcgatctctcgagcacttccgaatctctaccgagaagatgcccacctctctgatccacgctctggccctgaccaagcgagccgccgctaaggtgaacgaggacctgggcctgctgtctgaggaaaaggcctctgccatccgacaggccgccgacgaggtgctggctggacagcacgacgacgagttccctctggccatctggcagaccggctctggcacccagtctaacatgaacatgaacgaggttctggccaaccgagcctctgagctgctcggcggcgtgcgaggcatggaacgaaaggtgcaccccaacgacgacgtgaacaagtctcagtcctctaacgacgtgttccccaccgccatgcacgtggccgctctgctggccctgcgaaagcagctgattccccagctcaagaccctgactcagaccctgaacgagaagtctcgagccttcgccgacatcgtgaagatcggacgaacccacctccaggacgctacccctctgactctgggccaagagatctccggctgggtcgccatgctggaacacaacctgaagcacattgagtactcgctgccccacgtcgccgagctggccctcggcggcaccgccgtcggcaccggcctgaacactcaccccgagtacgcccgacgagtggccgacgagctggctgtgatcacctgtgctcccttcgtgaccgctcctaacaagttcgaggccctggccacctgtgacgccctggtgcaggcccacggcgccctgaagggcctcgccgcttctctgatgaagatcgccaacgacgtccgatggctggcctctggaccccgatgtggcatcggcgagatctctatccccgagaacgagcccggatcttctatcatgcccggcaaggtgaaccccactcagtgcgaggctctgaccatgctgtgctgccaggtgatgggcaacgacgtggccatcaacatgggcggagcctctggcaacttcgagctgaacgtgttccgacctatggtgatccacaactttctgcagtctgtgcgactgctggccgacggcatggaatctttcaacaagcactgtgccgtgggcatcgagcccaaccgagagcgaatcaaccagctgctgaacgagtctctgatgctggtcaccgctctgaacacccacatcggctacgacaaggccgctgagattgccaagaaggcccacaaggaaggactgaccctgaaggctgccgctctggctctgggatacctgtccgaggccgagttcgactcttgggtgcgacccgagcagatggtgggctctatgaaggccggacgataa

SEQ ID NO: 6 - DNA, 1317 bp, synthetic construct
  source 1..1317: mol_type = other DNA
atgggcgagctgaaggaaatcctgaagcagcgataccacgagctgctggactggaacgtgaaggcccctcacgtgcccctgtctcagcgactgaagcacttcacctggtcctggttcgcctgcaccatggccaccggcggagtgggcctgattatcggctctttccccttccgattctacggcctgaacaccatcggcaagatcgtgtatatcctgcagatcttcctgttctctctgttcggctcttgcatgctgttccgattcatcaagtacccctctaccatcaaggactcttggaaccaccacctcgagaagctgttcattgccacctgtctgctgtctatctctaccttcatcgacatgctggccatctacgcttaccccgacaccggtgagtggatggtgtgggtgatccgaatcctgtactacatctacgtggccgtgtctttcatctactgcgtgatggccttcttcaccatcttcaacaaccacgtgtacaccatcgagactgcttctcccgcctggattctgcctatcttccctcctatgatctgcggcgtgatcgctggcgccgtgaactctacccagcctgctcaccagctgaagaacatggtgatcttcggcatcctgttccaaggcctcggcttctgggtgtacctgctgctgttcgccgtcaacgtgctgcgattcttcaccgtcggcctggctaagccccaggaccgacctggcatgttcatgttcgtgggccctccagccttctctggactggccctgatcaacattgcccgaggcgccatgggctctcgaccctacattttcgtgggcgccaactcttctgagtacctgggcttcgtgtccaccttcatggccatcttcatctggggcctcgccgcctggtgctactgcctggctatggtgtctttcctggccggcttcttcactcgagcccctctgaagttcgcctgtggctggttcgctttcatcttccccaacgtgggattcgtgaactgcaccattgagatcggaaagatgatcgactctaaggccttccagatgttcggccacatcatcggagtgatcctgtgcatccagtggatcctgctgatgtacctgatggtgcgagccttcctggtgaacgacctgtgctaccccggcaaggacgaggacgctcaccctccacctaagcctaacaccggcgtgctgaaccccacctttccacctgagaaggctcccgcctctctcgagaaggttgacacccacgtgacctctaccggcggtgagtctgaccctccatcttctgagcacgagtctgtgtaa

SEQ ID NO: 7 - DNA, 720 bp, synthetic construct
  source 1..720: mol_type = other DNA
atggtgagcaagcagatcctgaagaacaccggcctgcaggagatcatgagcttcaaggtgaacctggagggcgtggtgaacaaccacgtgttcaccatggagggctgcggcaagggcaacatcctgttcggcaaccagctggtgcagatccgcgtgaccaagggcgcccccctgcccttcgccttcgacatcctgagccccgccttccagtacggcaaccgcaccttcaccaagtaccccgaggacatcagcgacttcttcatccagagcttccccgccggcttcgtgtacgagcgcaccctgcgctacgaggacggcggcctggtggagatccgcagcgacatcaacctgatcgaggggatgttcgtgtaccgcgtggagtacaagggccgcaacttccccaacgacggccccgtgatgaagaagaccatcaccggcctgcagcccagcttcgaggtggtgtacatgaacgacggcgtgctggtgggccaggtgatcctggtgtaccgcctgaacagcggcaagttctacagctgccacatgcgcaccctgatgaagagcaagggcgtggtgaaggacttccccgagtaccacttcatccagcaccgcctggagaagacctacgtggaggacggcggcttcgtagagcagcacgagaccgccatcgcccagctgaccagcctgggcaagcccctgggcagcctgcacgagtgggtgtaa

SEQ ID NO: 8 - DNA, 711 bp, synthetic construct
  source 1..711: mol_type = other DNA
atggtgagcaagggcgaggaggataacatggccatcatcaaggagttcatgcgcttcaaggtgcacatggagggctccgtgaacggccacgagttcgagatcgagggcgagggcgagggccgcccctacgagggcacccagaccgccaagctgaaggtgaccaagggtggccccctgcccttcgcctgggacatcctgtcccctcagttcatgtacggctccaaggcctacgtgaagcaccccgccgacatccccgactacttgaagctgtccttccccgagggcttcaagtgggagcgcgtgatgaacttcgaggacggcggcgtggtgaccgtgacccaggactcctccctgcaggacggcgagttcatctacaaggtgaagctgcgcggcaccaacttcccctccgacggccccgtaatgcagaagaagacgatgggctgggaggcctcctccgagcggatgtaccccgaggacggcgccctgaagggcgagatcaagcagaggctgaagctgaaggacggcggccactacgacgctgaggtcaagaccacctacaaggccaagaagcccgtgcagctgcccggcgcctacaacgtcaacatcaagttggacatcacctcccacaacgaggactacaccatcgtggaacagtacgaacgcgccgagggccgccactccaccggcggcatggacgagctgtacaagtag

SEQ ID NO: 9 - DNA, 69 bp, synthetic construct
  source 1..69: mol_type = other DNA
atgttcgccctgagaagatctctgctttccgcaggccgaatcgctcgaccccagcaggttgctcgattc

SEQ ID NO: 10 - protein, 23 aa, synthetic construct
MFALRRSLLSAGRIARPQQVARF

SEQ ID NO: 11 - DNA, 40 bp, synthetic construct
  source 1..40: mol_type = other DNA
ataagaatcattcaaaggttatggtggacggtcgatcttc

SEQ ID NO: 12 - DNA, 40 bp, synthetic construct
  source 1..40: mol_type = other DNA
acataactaattacatgattttaggagccagagggctcgg

SEQ ID NO: 13 - DNA, 39 bp, synthetic construct
  source 1..39: mol_type = other DNA
cagtactaaccgcagatttatgttccgaacccgagttac

SEQ ID NO: 14 - DNA, 39 bp, synthetic construct
  source 1..39: mol_type = other DNA
taactaattacatgaatttttaagggttctgcttgacaa

SEQ ID NO: 15 - DNA, 39 bp, synthetic construct
  source 1..39: mol_type = other DNA
attaaacacacatcaacagatgatgaacaccgtgcgatc

SEQ ID NO: 16 - DNA, 39 bp, synthetic construct
  source 1..39: mol_type = other DNA
gacaggccatggaggtacgttatcgtccggccttcatag

SEQ ID NO: 17 - DNA, 23 bp, synthetic construct
  source 1..23: mol_type = other DNA
aatttatctcattgtcactcaat

SEQ ID NO: 18 - DNA, 20 bp, synthetic construct
  source 1..20: mol_type = other DNA
tatttcgcgtctcggcctct

SEQ ID NO: 19 - DNA, 42 bp, synthetic construct
  source 1..42: mol_type = other DNA
aggccgagacgcgaaatagataacagggtaattatcgcttcg

SEQ ID NO: 20 - DNA, 43 bp, synthetic construct
  source 1..43: mol_type = other DNA
ttgcttggtggagtctggggatgattaccctgttatccctaca

SEQ ID NO: 21 - DNA, 19 bp, synthetic construct
  source 1..19: mol_type = other DNA
cccagactccaccaagcaa

SEQ ID NO: 22 - DNA, 31 bp, synthetic construct
  source 1..31: mol_type = other DNA
tcagcgagccgacggaaatgccgattcggaa

SEQ ID NO: 23 - DNA, 31 bp, synthetic construct
  source 1..31: mol_type = other DNA
ggcatttccggcgtctcgctgatccacgtgc

SEQ ID NO: 24 - DNA, 25 bp, synthetic construct
  source 1..25: mol_type = other DNA
gtgattttgaagtcttttacttgtg

SEQ ID NO: 25 - DNA, 39 bp, synthetic construct
  source 1..39: mol_type = other DNA
taagaatcattcaaaggttatgttcgccctgagaagatc

SEQ ID NO: 26 - DNA, 20 bp, synthetic construct
  source 1..20: mol_type = other DNA
gaatcgagcaacctgctggg

SEQ ID NO: 27 - DNA, 39 bp, synthetic construct
  source 1..39: mol_type = other DNA
ccagcaggttgctcgattcgtggacggtcgatcttccgc

SEQ ID NO: 28 - DNA, 38 bp, synthetic construct
  source 1..38: mol_type = other DNA
cagcaggttgctcgattcttcgccctgcgacgatctct

SEQ ID NO: 29 - DNA, 38 bp, synthetic construct
  source 1..38: mol_type = other DNA
ataactaattacatgattttagtacagcttggcaatgt

SEQ ID NO: 30 - DNA, 39 bp, synthetic construct
  source 1..39: mol_type = other DNA
ccagcaggttgctcgattcaagaagatgaacctggccgt

SEQ ID NO: 31 - DNA, 39 bp, synthetic construct
  source 1..39: mol_type = other DNA
cataactaattacatgattttagttcttcttagagtact

SEQ ID NO: 32 - DNA, 39 bp, synthetic construct
  source 1..39: mol_type = other DNA
attaaacacacatcaacagatgttccgaacccgagttac

SEQ ID NO: 33 - DNA, 39 bp, synthetic construct
  source 1..39: mol_type = other DNA
gacaggccatggaggtacgttaagggttctgcttgacaa

SEQ ID NO: 34 - DNA, 39 bp, synthetic construct
  source 1..39: mol_type = other DNA
attaaacacacatcaacagatggttaaagctgtcgttgc

SEQ ID NO: 35 - DNA, 39 bp, synthetic construct
  source 1..39: mol_type = other DNA
gacaggccatggaggtacgctagttggcaggaggagggt

SEQ ID NO: 36 - DNA, 39 bp, synthetic construct
  source 1..39: mol_type = other DNA
attaaacacacatcaacagatgaactctccccagaacgt

SEQ ID NO: 37 - DNA, 39 bp, synthetic construct
  source 1..39: mol_type = other DNA
gacaggccatggaggtacgttacagcagatctcgcacgg

SEQ ID NO: 38 - DNA, 39 bp, synthetic construct
  source 1..39: mol_type = other DNA
tttgcagtactaaccgcagttcgccctgagaagatctct

SEQ ID NO: 39 - DNA, 39 bp, synthetic construct
  source 1..39: mol_type = other DNA
cccagcaggttgctcgattcatgaacaccgtgcgatctg

SEQ ID NO: 40 - DNA, 39 bp, synthetic construct
  source 1..39: mol_type = other DNA
cataactaattacatgaatttatcgtccggccttcatag

SEQ ID NO: 41 - DNA, 39 bp, synthetic construct
  source 1..39: mol_type = other DNA
taagaatcattcaaaggttatgggcgagctgaaggaaat

SEQ ID NO: 42 - DNA, 40 bp, synthetic construct; identical to SEQ ID NO: 12
  source 1..40: mol_type = other DNA

SEQ ID NO: 43 - DNA, 39 bp, synthetic construct
  source 1..39: mol_type = other DNA
taagaatcattcaaaggttatggtgagcaagcagatcct

SEQ ID NO: 44 - DNA, 39 bp, synthetic construct
  source 1..39: mol_type = other DNA
cataactaattacatgattttacacccactcgtgcaggc

SEQ ID NO: 45 - DNA, 39 bp, synthetic construct
  source 1..39: mol_type = other DNA
actgcacacgacctcgctggtgagcaagggcgaggagga

SEQ ID NO: 46 - DNA, 39 bp, synthetic construct
  source 1..39: mol_type = other DNA
cataactaattacatgattctacttgtacagctcgtcca

SEQ ID NO: 47 - DNA, 21 bp, synthetic construct
  source 1..21: mol_type = other DNA
acgactcaacaagacacaaag

SEQ ID NO: 48 - DNA, 20 bp, synthetic construct
  source 1..20: mol_type = other DNA
acatgatggactcttcattg